European Patent Specification EP 3 463 388 B1, published September 11, 2024. Title: Particles with RNA Cleaving Nucleobase Polymers and Uses for Managing Inflammatory Disorders. Applicant: Emory University Salaita, Khalid Wongtrakool, Cherry. The sequence listing filed with the application follows.

SEQUENCE LISTING (55 sequences)

SEQ ID NO: 1 - DNA, 31 bp, Artificial
  Synthetic
tgggcttaaggctagctacaacgagaggggc

SEQ ID NO: 2 - DNA, 31 bp, Artificial
  Synthetic
tggtctgaggctagctacaacgaagttcgca

SEQ ID NO: 3 - DNA, 34 bp, Artificial
  Synthetic
gtctgttaataggctagctacaacgatgtgaagc

SEQ ID NO: 4 - DNA, 32 bp, Artificial
  Synthetic
tgctagacaggctagctacaacgattttcggt

SEQ ID NO: 5 - DNA, 33 bp, Artificial
  Synthetic
tttgctagaggctagctacaacgaatttttcgg

SEQ ID NO: 6 - DNA, 33 bp, Artificial
  Synthetic
ctttttggaggctagctacaacgattgctagac

SEQ ID NO: 7 - DNA, 34 bp, Artificial
  Synthetic
ttttttgcaggctagctacaacgatttttggatt

SEQ ID NO: 8 - DNA, 32 bp, Artificial
  Synthetic
gcttcatgaggctagctacaacgaactgctcc

SEQ ID NO: 9 - DNA, 32 bp, Artificial
  Synthetic
aggcttcaggctagctacaacgagatactgct

SEQ ID NO: 10 - DNA, 33 bp, Artificial
  Synthetic
ggcttattcaggctagctacaacgaagatgggg

SEQ ID NO: 11 - DNA, 33 bp, Artificial
  Synthetic
aatggcttaggctagctacaacgatcacagatg

SEQ ID NO: 12 - DNA, 33 bp, Artificial
  Synthetic
taggggataggctagctacaacgagagtcagaa

SEQ ID NO: 13 - DNA, 33 bp, Artificial
  Synthetic
aataggggaggctagctacaacgaatgagtcag

SEQ ID NO: 14 - DNA, 34 bp, Artificial
  Synthetic
cactagagaggctagctacaacgacctgttaaat

SEQ ID NO: 15 - DNA, 32 bp, Artificial
  Synthetic
tcacagcaggctagctacaacgatagagaccc

SEQ ID NO: 16 - DNA, 34 bp, Artificial
  Synthetic
ttttttttcaggctagctacaacgaagcactaga

SEQ ID NO: 17 - DNA, 34 bp, Artificial
  Synthetic
gttcagcaggctagctacaacgatttttttttca

SEQ ID NO: 18 - DNA, 36 bp, Artificial
  Synthetic
atataagttataggctagctacaacgagcaatgttc

SEQ ID NO: 19 - DNA, 36 bp, Artificial
  Synthetic
caatataagttaggctagctacaacgaatgcaatgt

SEQ ID NO: 20 - DNA, 33 bp, Artificial
  Synthetic
attccttaaaggctagctacaacgattcttggc

SEQ ID NO: 21 - DNA, 33 bp, Artificial
  Synthetic
ggaaacaaaaggctagctacaacgatggcagtt

SEQ ID NO: 22 - DNA, 33 bp, Artificial
  Synthetic
gaaaggaaaggctagctacaacgaaaaactggc

SEQ ID NO: 23 - DNA, 35 bp, Artificial
  Synthetic
ttttcttttaaggctagctacaacgagcatcaaac

SEQ ID NO: 24 - DNA, 33 bp, Artificial
  Synthetic
acaacaattaggctagctacaacgaagggactt

SEQ ID NO: 25 - DNA, 34 bp, Artificial
  Synthetic
caaacaacaaggctagctacaacgatacagggac

SEQ ID NO: 26 - DNA, 35 bp, Artificial
  Synthetic
atacaaacaaggctagctacaacgaaattacaggg

SEQ ID NO: 27 - DNA, 35 bp, Artificial
  Synthetic
tacatacaaaggctagctacaacgaaacaattaca

SEQ ID NO: 28 - DNA, 35 bp, Artificial
  Synthetic
tgaattatacaggctagctacaacgaacaaacaac

SEQ ID NO: 29 - DNA, 36 bp, Artificial
  Synthetic
tttgaattataggctagctacaacgaatacaaacaa

SEQ ID NO: 30 - DNA, 33 bp, Artificial
  Synthetic
tcttttcttaggctagctacaacgatttggtgc

SEQ ID NO: 31 - DNA, 37 bp, Artificial
  Synthetic
ataaatctacaggctagctacaacgacttttcttatt

SEQ ID NO: 32 - DNA, 36 bp, Artificial
  Synthetic
aaataaatctaggctagctacaacgaatcttttctt

SEQ ID NO: 33 - DNA, 38 bp, Artificial
  Synthetic
tgtataatatgaggctagctacaacgagaaataaatct

SEQ ID NO: 34 - DNA, 37 bp, Artificial
  Synthetic
tctgtataataggctagctacaacgagatgaaataaa

SEQ ID NO: 35 - DNA, 35 bp, Artificial
  Synthetic
gtctgtataaggctagctacaacgaatgatgaaat

SEQ ID NO: 36 - DNA, 34 bp, Artificial
  Synthetic
aatttatacaaggctagctacaacgaagttcggt

SEQ ID NO: 37 - DNA, 37 bp, Artificial
  Synthetic
aaataaatttataggctagctacaacgaaacagttcg

SEQ ID NO: 38 - DNA, 36 bp, Artificial
  Synthetic
taaataaatttaggctagctacaacgaacaacagtt

SEQ ID NO: 39 - DNA, 36 bp, Artificial
  Synthetic
cagtaaataaaggctagctacaacgattatacaaca

SEQ ID NO: 40 - DNA, 35 bp, Artificial
  Synthetic
agcagtaaaggctagctacaacgaaaatttataca

SEQ ID NO: 41 - DNA, 34 bp, Artificial
  Synthetic
gttcttaagaggctagctacaacgatagcagtaa

SEQ ID NO: 42 - DNA, 34 bp, Artificial
  Synthetic
caaccaaaaaggctagctacaacgatgagagaga

SEQ ID NO: 43 - DNA, 37 bp, Artificial
  Synthetic
ttagaagctaggctagctacaacgattaataaatatc

SEQ ID NO: 44 - DNA, 32 bp, Artificial
  Synthetic
tgacatgcaggctagctacaacgagctggtag

SEQ ID NO: 45 - DNA, 32 bp, Artificial
  Synthetic
tcactaacaggctagctacaacgaagaacacg

SEQ ID NO: 46 - DNA, 34 bp, Artificial
  Synthetic
tgatcactaaggctagctacaacgaacagaacac

SEQ ID NO: 47 - DNA, 35 bp, Artificial
  Synthetic
attattccaaggctagctacaacgaagactgtatt

SEQ ID NO: 48 - DNA, 38 bp, Artificial
  Synthetic
aaatattttcaggctagctacaacgatttattattatg

SEQ ID NO: 49 - DNA, 36 bp, Artificial
  Synthetic
tagttttaaaaggctagctacaacgaattttcactt

SEQ ID NO: 50 - DNA, 32 bp, Artificial
  Synthetic
tggatggaggctagctacaacgagtcttggag

SEQ ID NO: 51 - DNA, 15 bp, Artificial
  Synthetic
ggctagctacaacga

SEQ ID NO: 52 - DNA, 3069 bp, Homo sapiens
ggcgccgtcttgatactttcagaaagaatgcattccctgtaaaaaaaaaaaaaaaatactgagagagggagagagagagagaagaagagagagagacggagggagagcgagacagagcgagcaacgcaatctgaccgagcaggtcgtacgccgccgcctcctcctcctctctgctcttcgctacccaggtgacccgaggagggactccgcctccgagcggctgaggaccccggtgcagaggagcctggctcgcagaattgcagagtcgtcgcccctttttacaacctggtcccgttttattctgccgtacccagtttttggatttttgtcttccccttcttctctttgctaaacgacccctccaagataatttttaaaaaaccttctcctttgctcacctttgcttcccagccttcccatccccccaccgaaagcaaatcattcaacgacccccgaccctccgacggcaggagccccccgacctcccaggcggaccgccctccctccccgcgcgcgggttccgggcccggcgagagggcgcgagcacagccgaggccatggaggtgacggcggaccagccgcgctgggtgagccaccaccaccccgccgtgctcaacgggcagcacccggacacgcaccacccgggcctcagccactcctacatggacgcggcgcagtacccgctgccggaggaggtggatgtgctttttaacatcgacggtcaaggcaaccacgtcccgccctactacggaaactcggtcagggccacggtgcagaggtaccctccgacccaccacgggagccaggtgtgccgcccgcctctgcttcatggatccctaccctggctggacggcggcaaagccctgggcagccaccacaccgcctccccctggaatctcagccccttctccaagacgtccatccaccacggctccccggggcccctctccgtctaccccccggcctcgtcctcctccttgtcggggggccacgccagcccgcacctcttcaccttcccgcccaccccgccgaaggacgtctccccggacccatcgctgtccaccccaggctcggccggctcggcccggcaggacgagaaagagtgcctcaagtaccaggtgcccctgcccgacagcatgaagctggagtcgtcccactcccgtggcagcatgaccgccctgggtggagcctcctcgtcgacccaccaccccatcaccacctacccgccctacgtgcccgagtacagctccggactcttcccccccagcagcctgctgggcggctcccccaccggcttcggatgcaagtccaggcccaaggcccggtccagcacagaaggcagggagtgtgtgaactgtggggcaacctcgaccccactgtggcggcgagatggcacgggacactacctgtgcaacgcctgcgggctctatcacaaaatgaacggacagaaccggcccctcattaagcccaagcgaaggctgtctgcagccaggagagcagggacgtcctgtgcgaactgtcagaccaccacaaccacactctggaggaggaatgccaatggggaccctgtctgcaatgcctgtgggctctactacaagcttcacaatattaacagacccctgactatgaagaaggaaggcatccagaccagaaaccgaaaaatgtctagcaaatccaaaaagtgcaaaaaagtgcatgactcactggaggacttccccaagaacagctcgtttaacccggccgccctctccagacacatgtcctccctgagccacatctcgcccttcagccactccagccacatgctgaccacgcccacgccgatgcacccgccatccagcctgtcctttggaccacaccacccctccagcatggtcaccgccatgggttagagccctgctcgatgctcacagggcccccagcgagagtccctgcagtccctttcgacttgcatttttgcaggagcagtatcatgaagcctaaacgcgatggatatatgtttttgaaggcagaaagcaaaattatgtttgccactttgcaaaggagctcactgtggtgtctgtgttccaaccactgaatctggaccccatctgtgaataagccattctgactcatatcccctatttaacagggtctctagtgctgtgaaaaaaaaaatgctgaacattgcatataacttatattgtaagaaatactgtacaatgactttattgcatctgggtagctgtaaggcatgaaggatgccaagaagtttaaggaatatgggagaaatagtgtggaaattaagaagaaactaggtctgatattcaaatggacaaactgccagttttgtttcctttcactggccacagttgtttgatgcattaaaagaaaataaaaaaaagaaaaaagagaaaagaaaaaaaaagaaaaaagttgtaggcgaatcatttgttcaaagctgttggcctctgcaaaggaaataccagttctgggcaatcagtgttaccgttcaccagttgccgttgagggtttcagagagcctttttctaggcctacatgctttgtgaacaagtccctgtaattgttgtttgtatgtataattcaaagcaccaaaataagaaaagatgtagatttatttcatcatattatacagaccgaactgttgtataatttatttactgctagtcttaagaactgctttctttcgtttgtttgtttcaatattttccttctctctcaatttttggttgaataaactagattacattcagttggcctaaggtggttgtgctcggagggtttcttgtttcttttccattttgtttttggatgatatttattaaatagcttctaagagtccggcggcatctgtcttgtccctattcctgcagcctgtgctgagggtagcagtgtatgagctaccagcgtgcatgtcagcgaccctggcccgacaggccacgtcctgcaatcggcccggctgcctcttcgccctgtcgtgttctgtgttagtgatcactgcctttaatacagtctgttggaataatattataagcataataataaagtgaaaatattttaaaactacaa

SEQ ID NO: 53 - DNA, 33 bp, Artificial
  Synthetic
gtggatggaggctagctacaacgagtcttggag

SEQ ID NO: 54 - DNA, 31 bp, Artificial
  Synthetic
tggatggaggctagctacaacgagtcttgga

SEQ ID NO: 55 - DNA, 29 bp, Artificial
  Synthetic
ggatggaggctagctacaacgagtcttgg